European Patent Application EP 4 644 409 A1, published November 5, 2025. Title: SWEET-TASTING PROTEIN BRAZZEIN MUTANT HAVING HIGH SWEETNESS AND PREPARATION METHOD THEREFOR. Applicant: Nanjing Bestzyme Bio-Engineering Co., Ltd. The sequence listing filed with the application follows.

SEQUENCE LISTING (44 sequences)

SEQ ID NO: 1 - protein, 53 aa, Pentadiplandra brazzeana
DKCKKVYENYPVSKCQLANQCNYDCKLDKHARSGECFYDEKRNLQCICDYCEY

SEQ ID NO: 2 - DNA, 159 bp, Pentadiplandra brazzeana
  source 1..159: mol_type = genomic DNA
gacaagtgcaagaaggtctacgagaactaccctgtctccaagtgccagctcgccaaccagtgcaactacgattgcaagctcgataagcacgcccgctccggcgagtgcttctacgatgagaagcgcaacctccagtgcatctgcgactactgcgagtac

SEQ ID NO: 3 - protein, 53 aa, synthetic construct
DKCKKVYENYPVSKCQLANQCNYDCKLDKHARSGDCFYDAKRNLQCICDYCEY

SEQ ID NO: 4 - DNA, 159 bp, synthetic construct
  source 1..159: mol_type = other DNA
gacaagtgcaagaaggtctacgagaactaccccgtctccaagtgccagctcgccaaccagtgcaactacgactgcaagctcgacaagcacgcccgctccggtgactgcttctacgacgccaagcgcaacctccagtgcatctgcgactactgcgagtac

SEQ ID NO: 5 - protein, 53 aa, synthetic construct
DKCKKVYENYPVSKCQLANQCNYDCKLDKHARSGDCFYDDKRNLQCICDYCEY

SEQ ID NO: 6 - DNA, 159 bp, synthetic construct
  source 1..159: mol_type = other DNA
gacaagtgcaagaaggtctacgagaactaccccgtctccaagtgccagctcgccaaccagtgcaactacgactgcaagctcgacaagcacgcccgctccggtgactgcttctacgacgacaagcgcaacctccagtgcatctgcgactactgcgagtac

SEQ ID NO: 7 - protein, 53 aa, synthetic construct
DKCKKVYENYPVSKCQLANQCNYDCKLDKHARSGDCFYDKKRNLQCICDYCEY

SEQ ID NO: 8 - DNA, 159 bp, synthetic construct
  source 1..159: mol_type = other DNA
gacaagtgcaagaaggtctacgagaactaccccgtctccaagtgccagctcgccaaccagtgcaactacgactgcaagctcgacaagcacgcccgctccggtgactgcttctacgacaagaagcgcaacctccagtgcatctgcgactactgcgagtac

SEQ ID NO: 9 - protein, 53 aa, synthetic construct
DKCKKVYENYPVSKCQLANQCNYDCKLDKHARSGDCFYDRKRNLQCICDYCEY

SEQ ID NO: 10 - DNA, 159 bp, synthetic construct
  source 1..159: mol_type = other DNA
gacaagtgcaagaaggtctacgagaactaccccgtctccaagtgccagctcgccaaccagtgcaactacgactgcaagctcgacaagcacgcccgctccggtgactgcttctacgaccgcaagcgcaacctccagtgcatctgcgactactgcgagtac

SEQ ID NO: 11 - protein, 53 aa, synthetic construct
DKCKKVYENYPVSKCQLANQCNYDCKLDKRARSGDCFYDAKRNLQCICDYCEY

SEQ ID NO: 12 - DNA, 159 bp, synthetic construct
  source 1..159: mol_type = other DNA
gacaagtgcaagaaggtctacgagaactaccccgtctccaagtgccagctcgccaaccagtgcaactacgactgcaagctcgacaagcgcgcccgctccggtgactgcttctacgacgccaagcgcaacctccagtgcatctgcgactactgcgagtac

SEQ ID NO: 13 - protein, 53 aa, synthetic construct
DKCKKVYENYPVSKCQLANQCNYDCKLDKRARSGDCFYDKKRNLQCICDYCEY

SEQ ID NO: 14 - DNA, 159 bp, synthetic construct
  source 1..159: mol_type = other DNA
gacaagtgcaagaaggtctacgagaactaccccgtctccaagtgccagctcgccaaccagtgcaactacgactgcaagctcgacaagcgcgcccgctccggtgactgcttctacgacaagaagcgcaacctccagtgcatctgcgactactgcgagtac

SEQ ID NO: 15 - protein, 53 aa, synthetic construct
DKCKKVYENYPVSKCQLANQCNYDCKLDKRARSGDCFYDRKRNLQCICDYCEY

SEQ ID NO: 16 - DNA, 159 bp, synthetic construct
  source 1..159: mol_type = other DNA
gacaagtgcaagaaggtctacgagaactaccccgtctccaagtgccagctcgccaaccagtgcaactacgactgcaagctcgacaagcgcgcccgctccggtgactgcttctacgaccgcaagcgcaacctccagtgcatctgcgactactgcgagtac

SEQ ID NO: 17 - protein, 28 aa, synthetic construct
DDNLVGGMTLDLPSDAPPISLSSSTNSA

SEQ ID NO: 18 - protein, 6 aa, synthetic construct
VALEKR

SEQ ID NO: 19 - protein, 87 aa, synthetic construct
DDNLVGGMTLDLPSDAPPISLSSSTNSAVALEKRDKCKKVYENYPVSKCQLANQCNYDCKLDKHARSGECFYDEKRNLQCICDYCEY

SEQ ID NO: 20 - DNA, 261 bp, synthetic construct
  source 1..261: mol_type = other DNA
gatgataacctcgtcggcggcatgaccctcgatctcccttccgatgctcctcctatcagcctctcctcctccaccaactccgccgtcgctctcgagaagcgcgacaagtgcaagaaggtctacgagaactaccctgtctccaagtgccagctcgccaaccagtgcaactacgattgcaagctcgataagcacgcccgctccggcgagtgcttctacgatgagaagcgcaacctccagtgcatctgcgactactgcgagtac

SEQ ID NO: 21 - protein, 87 aa, synthetic construct
DDNLVGGMTLDLPSDAPPISLSSSTNSAVALEKRDKCKKVYENYPVSKCQLANQCNYDCKLDKHARSGDCFYDAKRNLQCICDYCEY

SEQ ID NO: 22 - DNA, 261 bp, synthetic construct
  source 1..261: mol_type = other DNA
gatgataacctcgtcggcggcatgaccctcgatctcccttccgatgctcctcctatcagcctctcctcctccaccaactccgccgtcgctctcgagaagcgcgacaagtgcaagaaggtctacgagaactaccccgtctccaagtgccagctcgccaaccagtgcaactacgactgcaagctcgacaagcacgcccgctccggtgactgcttctacgacgccaagcgcaacctccagtgcatctgcgactactgcgagtac

SEQ ID NO: 23 - protein, 87 aa, synthetic construct
DDNLVGGMTLDLPSDAPPISLSSSTNSAVALEKRDKCKKVYENYPVSKCQLANQCNYDCKLDKHARSGDCFYDDKRNLQCICDYCEY

SEQ ID NO: 24 - DNA, 261 bp, synthetic construct
  source 1..261: mol_type = other DNA
gatgataacctcgtcggcggcatgaccctcgatctcccttccgatgctcctcctatcagcctctcctcctccaccaactccgccgtcgctctcgagaagcgcgacaagtgcaagaaggtctacgagaactaccccgtctccaagtgccagctcgccaaccagtgcaactacgactgcaagctcgacaagcacgcccgctccggtgactgcttctacgacgacaagcgcaacctccagtgcatctgcgactactgcgagtac

SEQ ID NO: 25 - protein, 87 aa, synthetic construct
DDNLVGGMTLDLPSDAPPISLSSSTNSAVALEKRDKCKKVYENYPVSKCQLANQCNYDCKLDKHARSGDCFYDKKRNLQCICDYCEY

SEQ ID NO: 26 - DNA, 261 bp, synthetic construct
  source 1..261: mol_type = other DNA
gatgataacctcgtcggcggcatgaccctcgatctcccttccgatgctcctcctatcagcctctcctcctccaccaactccgccgtcgctctcgagaagcgcgacaagtgcaagaaggtctacgagaactaccccgtctccaagtgccagctcgccaaccagtgcaactacgactgcaagctcgacaagcacgcccgctccggtgactgcttctacgacaagaagcgcaacctccagtgcatctgcgactactgcgagtac

SEQ ID NO: 27 - protein, 87 aa, synthetic construct
DDNLVGGMTLDLPSDAPPISLSSSTNSAVALEKRDKCKKVYENYPVSKCQLANQCNYDCKLDKHARSGDCFYDRKRNLQCICDYCEY

SEQ ID NO: 28 - DNA, 261 bp, synthetic construct
  source 1..261: mol_type = other DNA
gatgataacctcgtcggcggcatgaccctcgatctcccttccgatgctcctcctatcagcctctcctcctccaccaactccgccgtcgctctcgagaagcgcgacaagtgcaagaaggtctacgagaactaccccgtctccaagtgccagctcgccaaccagtgcaactacgactgcaagctcgacaagcacgcccgctccggtgactgcttctacgaccgcaagcgcaacctccagtgcatctgcgactactgcgagtac

SEQ ID NO: 29 - protein, 87 aa, synthetic construct
DDNLVGGMTLDLPSDAPPISLSSSTNSAVALEKRDKCKKVYENYPVSKCQLANQCNYDCKLDKRARSGDCFYDAKRNLQCICDYCEY

SEQ ID NO: 30 - DNA, 261 bp, synthetic construct
  source 1..261: mol_type = other DNA
gatgataacctcgtcggcggcatgaccctcgatctcccttccgatgctcctcctatcagcctctcctcctccaccaactccgccgtcgctctcgagaagcgcgacaagtgcaagaaggtctacgagaactaccccgtctccaagtgccagctcgccaaccagtgcaactacgactgcaagctcgacaagcgcgcccgctccggtgactgcttctacgacgccaagcgcaacctccagtgcatctgcgactactgcgagtac

SEQ ID NO: 31 - protein, 87 aa, synthetic construct
DDNLVGGMTLDLPSDAPPISLSSSTNSAVALEKRDKCKKVYENYPVSKCQLANQCNYDCKLDKRARSGDCFYDKKRNLQCICDYCEY

SEQ ID NO: 32 - DNA, 261 bp, synthetic construct
  source 1..261: mol_type = other DNA
gatgataacctcgtcggcggcatgaccctcgatctcccttccgatgctcctcctatcagcctctcctcctccaccaactccgccgtcgctctcgagaagcgcgacaagtgcaagaaggtctacgagaactaccccgtctccaagtgccagctcgccaaccagtgcaactacgactgcaagctcgacaagcgcgcccgctccggtgactgcttctacgacaagaagcgcaacctccagtgcatctgcgactactgcgagtac

SEQ ID NO: 33 - protein, 87 aa, synthetic construct
DDNLVGGMTLDLPSDAPPISLSSSTNSAVALEKRDKCKKVYENYPVSKCQLANQCNYDCKLDKRARSGDCFYDRKRNLQCICDYCEY

SEQ ID NO: 34 - DNA, 261 bp, synthetic construct
  source 1..261: mol_type = other DNA
gatgataacctcgtcggcggcatgaccctcgatctcccttccgatgctcctcctatcagcctctcctcctccaccaactccgccgtcgctctcgagaagcgcgacaagtgcaagaaggtctacgagaactaccccgtctccaagtgccagctcgccaaccagtgcaactacgactgcaagctcgacaagcgcgcccgctccggtgactgcttctacgaccgcaagcgcaacctccagtgcatctgcgactactgcgagtac

SEQ ID NO: 35 - DNA, 25 bp, synthetic construct
  source 1..25: mol_type = other DNA
taaatttttatatggcgggtggtgg

SEQ ID NO: 36 - DNA, 33 bp, synthetic construct
  source 1..33: mol_type = other DNA
gacgaggttatcatcagccaaagcaggtgccgc

SEQ ID NO: 37 - DNA, 33 bp, synthetic construct
  source 1..33: mol_type = other DNA
cttcttgcacttgtcagccaaagcaggtgccgc

SEQ ID NO: 38 - DNA, 38 bp, synthetic construct
  source 1..38: mol_type = other DNA
tactgcgagtactagagggtggagagtatatgatggta

SEQ ID NO: 39 - DNA, 35 bp, synthetic construct
  source 1..35: mol_type = other DNA
cttcgaagagatacaagtaagtgatggatcgcact

SEQ ID NO: 40 - DNA, 37 bp, synthetic construct
  source 1..37: mol_type = other DNA
gatccatcacttacttgtatctcttcgaagatgccga

SEQ ID NO: 41 - DNA, 18 bp, synthetic construct
  source 1..18: mol_type = other DNA
gggtgcgccatgataaac

SEQ ID NO: 42 - DNA, 33 bp, synthetic construct
  source 1..33: mol_type = other DNA
gcacctgctttggctgatgataacctcgtcggc

SEQ ID NO: 43 - DNA, 36 bp, synthetic construct
  source 1..36: mol_type = other DNA
gcacctgctttggctgacaagtgcaagaaggtctac

SEQ ID NO: 44 - DNA, 36 bp, synthetic construct
  source 1..36: mol_type = other DNA
tatactctccaccctctagtactcgcagtagtcgca